European Patent Application EP 4 141 124 A1, published March 1, 2023. Title: Verfahren zur biotechnologischen Herstellung von Aldehydgemischen. Applicant: Symrise AG. The sequence listing filed with the application follows.

SEQUENCE LISTING (15 sequences)

SEQ ID NO: 1 - protein, 587 aa, Leptolyngbya sp. PC 7375
MFDNFWHKLPTPLALLQLLKLRNDLREKNLHDTSQLPDSGELPKPQPSSDGSHLTARTADGSFNDLQQPQMGMAGTRFGRNVALGAVEAEAVPKLMTPNPREVSRILMTRDRFQPATMLNLLAAAWIQFENHDWFSHGDNEPDDQLEIPLEPHDPWPEEHRPMVVGKTLADKSRPDGARPKTFINTVTHWWDGSQIYGSDPETVDKLRSHVHGKLTIQDDGLLPVDPETGLDVTGFNDNWWIGLSMLHTVFTKEHNAICDHLKQEYPHWSDDILFNHARLINAALMAKIHTVEWTPAILPLPVTDIALNVNWSGFLGEDLKQVLGSVGEGELTDLLSGIVGSETDHHTAPYYLTEEFASVYRMHPLIPDELQFYSLDNNQPLQSADFFQISGKRSRTLLESIPMPDLYYSFGVAHPGEISLHNYPRSLQQLVRDNGEVFDLAAVDILRDRERGVPRYNRFRELIGRTRVKSFEEISSNQQWVEEMRRVYYNDINSVDLMVGLFAEDKPEGFGFSDTAFRVFILMASRRLKSDRFFTKDYRAEVYTQLGLDWIANNTMVTVLQRHFPTLAPALYDIDNAFKPWRRIGT

SEQ ID NO: 2 - protein, 584 aa, Calotrix sp. PCC 6303
MFGIPWHKLPTPLGLLKVVQFRGRLRKNNLQDTSQLADTTKLPETMKCPYHNYLKARTPDGSYNDLKHPEMGMVGTRFGRNIPLEDVKVDEANLLTPNPRTVSRMLLAREEFQPATILNLLAAAWIQFQTHDWFSHGNNQPDNKFQIPIDADDSWPQEHRPMEVSRTLEDPTRSGDTKNPATFINHCTHWWDGSQVYGNDKKTIEEVRSRVNGKMRLEEDGFLPLDPKLGIDKVGFPGAWWVGLSMLHTLFVKEHNTICDHLSKLYPEWKDDELFDHARLINAALMAKIHTVEWTPAILPHPVTDIALNANWWGILGQQVKDTVGHIGDSELLSGIIGSPTDHHAAPYYLTEEFVSVYRMHALIPDDFDFYSLKTRKLLHKKSFPEVAGSKTRAFMEEVQMSDLFYSFGISHPGAVRLHNYPKFLRQLTGELTGDPNGAFDLAAVDILRDRERGVPRYNRFRELIGRGKVKSFEEITSNKQWAKELREVYNNNIDSVDLMVGLYAEDIPEKFGFSDTAFRVFILMASRRLKSDRFFTKDYTAEVYTQFGLDWIDRNNLVTVLKRHHPELAPVLVNVTNGFKPWK

SEQ ID NO: 3 - DNA, 1764 bp, Leptolyngbya sp. PC 7375
atgttcgataacttctggcataaactgccgaccccgctggcactgctgcagctgctgaaactgcgcaatgatctgcgtgaaaaaaatctgcatgataccagtcagctgccggatagcggcgaactgccgaaaccgcagccgagtagtgatggcagtcatctgaccgcacgcaccgccgatggtagcttcaatgatctgcagcagccgcagatgggcatggcaggtacccgcttcggtcgcaatgtggcactgggtgccgttgaagccgaagcagtgccgaaactgatgaccccgaatccgcgtgaagttagtcgtattctgatgacccgtgatcgcttccagccggcaaccatgctgaatctgctggcagcagcatggattcagttcgaaaatcatgattggttcagtcatggcgataatgaaccggatgatcagctggaaattccgctggaaccgcatgatccgtggccggaagaacatcgtccgatggttgttggcaaaaccttagcagataaaagtcgtccggatggcgcacgcccgaaaaccttcattaataccgttacccattggtgggatggcagtcagatctatggtagcgatccggaaaccgtggataaactgcgtagtcatgttcatggcaaactgaccattcaggatgatggtctgctgccggttgatccggaaacaggcctggatgttaccggcttcaatgataattggtggattggcctgagtatgctgcataccgtgttcaccaaagaacataatgcaatctgtgatcatctgaaacaggaatatccgcattggagtgatgatattctgttcaatcatgcacgtctgattaatgccgcactgatggcaaaaattcataccgttgaatggaccccggccattctgccgctgccggtgaccgatattgcactgaatgtgaattggagtggcttcctgggtgaagatctgaaacaggttctgggcagcgtgggcgaaggtgaactgaccgatctgctgagtggcattgttggcagcgaaaccgatcatcataccgcaccgtattatctgaccgaagaattcgccagcgtgtatcgtatgcatccgctgattccggatgaactgcagttctatagcctggataataatcagccgctgcagagcgcagacttcttccagattagcggtaaacgtagccgtaccctgctggaaagcattccgatgccggatctgtattatagcttcggtgttgcccatccgggcgaaattagtctgcataattatccgcgcagcctgcagcagctggtgcgtgataatggtgaagtgttcgatctggccgccgtggatattctgcgcgatcgtgaacgtggtgtgccgcgctataatcgcttccgcgaactgattggccgcacccgtgttaaaagcttcgaagaaattagtagcaatcagcagtgggtggaagaaatgcgtcgcgtgtattataatgatattaatagtgtggacctgatggttggtctgttcgcagaagataaaccggaaggcttcggcttcagcgataccgccttccgcgtgttcattctgatggccagtcgtcgtctgaaaagtgatcgcttcttcaccaaagattatcgcgcagaagtgtatacccagctgggcctggattggattgccaataataccatggttaccgtgctgcagcgtcacttcccgaccctggcaccggcactgtatgatattgataatgcattcaaaccgtggcgtcgtattggtacctaa

SEQ ID NO: 4 - DNA, 1755 bp, Calotrix sp. PCC 6303
atgttcggcattccgtggcataaactgccgaccccgctgggtctgctgaaagttgtgcagttccgcggtcgtctgcgtaaaaataatctgcaggataccagtcagctggccgataccaccaaactgccggaaaccatgaaatgcccgtatcataattatctgaaagcacgcaccccggatggcagttataatgatctgaaacatccggaaatgggcatggttggcacccgcttcggccgtaatattccgctggaagatgttaaagttgatgaagcaaatctgctgaccccgaatccgcgcaccgtgagccgtatgctgctggcccgcgaagaattccagccggcaaccattctgaatctgctggcagcagcctggattcagttccagacccatgattggttcagtcatggtaataatcagccggataataaattccagattccgattgatgccgatgatagctggccgcaggaacatcgcccgatggaagttagccgtaccctggaagatccgacccgtagtggcgataccaaaaatccggccaccttcattaatcattgcacccattggtgggatggtagccaggtgtatggcaatgataaaaaaaccattgaagaggtgcgcagtcgtgttaatggcaaaatgcgtctggaagaagatggcttcctgccgctggatccgaaactgggcattgataaagtgggcttcccgggtgcatggtgggtgggcctgagcatgctgcataccctgttcgtgaaagaacataataccatctgtgatcatctgagtaaactgtatccggaatggaaagatgatgaactgttcgatcatgcacgtctgattaatgcagcactgatggccaaaattcataccgtggaatggaccccggccattctgccgcatccggtgaccgatattgcactgaatgccaattggtggggtattctgggccagcaggttaaagataccgtgggtcatattggcgatagtgaactgctgagcggtattattggcagcccgaccgatcatcatgcagccccgtattatctgaccgaagaattcgtgagcgtgtatcgtatgcatgccctgattccggatgacttcgacttctatagtctgaaaaccagaaaactgctgcataaaaaaagcttcccggaagtggcaggcagtaaaaccagagccttcatggaagaagttcagatgagtgatctgttctatagcttcggcattagccatccgggtgccgtgcgtctgcataattatccgaaattcctgcgtcagctgaccggtgaactgaccggcgatccgaatggtgcattcgatctggccgcagttgatattctgcgtgatcgtgaacgtggcgtgccgcgttataatcgcttccgtgaactgattggtcgtggtaaagttaaaagcttcgaagaaattaccagcaataaacagtgggccaaagaactgcgtgaagtgtataataataacattgatagcgtggatctgatggttggtctgtatgccgaagatattccggaaaaattcggcttcagtgataccgccttccgtgtgttcattctgatggccagtcgtcgtctgaaaagcgatcgcttcttcaccaaagattataccgcagaagtgtatacccagttcggtctggattggattgatcgcaataatctggtgaccgtgctgaaacgccatcatccggaactggcaccggttctggttaatgtgaccaatggcttcaaaccgtggaaataa

SEQ ID NO: 5 - protein, 452 aa, Lactobacillus sanfranciscensis
MKVIVVGCTHAGTFAVKQTIADHPDADVTVYEMNDNISFLSCGIALYLGKEIKNNDPRGLFYSSPEELSNLGANVQMRHQVTNVDPETKTIKVKDLITNEEKTEAYDKLIMTTGSKPTVPPIPGIDSSRVYLCKNYNDAKKLFEEAPKAKTITIIGSGYIGAELAEAYSNQNYNVNLIDGHERVLYKYFDKEFTDILAKDYEAHGVNLVLGSKVAAFEEVDDEIITKTLDGKEIKSDIAILCIGFRPNTELLKGKVAMLDNGAIITDEYMHSSNRDIFAAGDSAAVHYNPTNSNAYIPLATNAVRQGRLVGLNLTEDKVKDMGTQSSSGLKLYGRTYVSTGINTALAKANNLKVSEVIIADNYRPEFMLSTDEVLMSLVYDPKTRVILGGALSSMHDVSQSANVLSVCIQNKNTIDDLAMVDMLFQPQFDRPFNYLNILGQAAQAQADKAHK

SEQ ID NO: 6 - protein, 451 aa, Lactobacillus brevis
MKVTVVGCTHAGTFAIKQILAEHPDAEVTVYEKNDNISFLSCGIALYLGGKVADPQGLFYSSPEELKSLGANVQMNHNVLNIDPDQKTVTVENMNTHEQTTADYDKLVMTSGSWPIVPKIPGIDGDHVKLCKNWNHAQTLIEDAKSAKHITVIGAGYIGAELAEAYSTTGHDVTLIDAMDRVMPKYFDSEFTDVIEQDYRDNNVQLALGETVQSFTDTGDGVTIKTDKGSYDTNLAILCIGFRPNTGLLKGKVDMAKNGAIITDDYMRSSNPDIFAAGDSAAVHYNPTHQNAYIPLATNAVRQGILVGKNLVKPTVKYMGTQSSSGLALYDRTIVSTGLTLAAAKQQGINAEQVIVKDNYRPEFMPTTEPVLMSLVFDPDSRRILGGALMSRYDVSQSANTLSVCIQNENTIDDLAMVDMLFQPNFDRPFNYLNILAQAAQEKVAKFQPAE

SEQ ID NO: 7 - DNA, 1359 bp, Lactobacillus sanfranciscensis
atgaaagttattgtagtaggttgtactcacgctggcacttttgcagttaagcaaacgattgccgatcaccccgatgcagatgtgactgtatatgaaatgaatgataacatttcctttttatcatgtggaatcgccctttacttaggtaaagaaattaaaaacaatgatccccgagggcttttctactcaagtccagaagaattaagcaatcttggagctaacgtccaaatgcgtcatcaagttacaaacgttgatccagaaacaaaaacaatcaaagttaaagatttaatcaccaacgaagaaaaaacagaagcatatgacaaattaattatgaccactggttctaagcctactgttcctccaatccctggaatcgatagtagtcgcgtttacctttgtaaaaactataacgatgctaaaaagttatttgaagaagctcccaaagctaaaacgattactatcattggttctggttatattggtgccgaactggctgaagcctactcaaaccaaaattataacgttaatttaattgatggtcatgaacgagttctttacaagtattttgataaagaatttactgatattttagccaaagattatgaagctcatggtgttaacctggttcttggttcaaaagtagctgcttttgaagaagtcgatgatgaaattatcactaaaaccctagatggtaaagaaattaaatctgatattgcaattctttgtatcggtttccgccctaacactgaattacttaaaggtaaagttgccatgttggataacggtgcaatcattactgatgaatacatgcattcatcaaatcgcgacatttttgctgctggtgatagtgccgccgttcactacaaccccactaattctaacgcctacattcctttagctaccaacgccgtacgccaagggagattagttggcctaaatctgactgaagacaaagtaaaagacatgggaacccaatcttcatctggtcttaaactatacggtcggacttatgtctcaactggaatcaatacggctcttgctaaagccaataatttaaaagttagcgaagtaatcatagctgataattatcgtccagaatttatgttatcaacggatgaagttttaatgtcattagtgtatgatcctaagactcgtgtaattttgggaggggcgctttcaagtatgcacgatgtttcgcaatcagcgaacgtcttatcagtatgtattcaaaataaaaacacgattgacgatttagcaatggtggatatgttattccaaccacaatttgatcgtccgtttaactacttaaacattctaggccaagctgctcaagcacaagctgacaaagcacataaataa

SEQ ID NO: 8 - DNA, 1356 bp, Lactobacillus brevis
atgaaagtgaccgtggtgggctgcacccatgcgggcacctttgcgattaaacagattctggcggaacatccggatgcggaagtgaccgtgtatgaaaaaaacgataacattagctttctgagctgcggcattgcgctgtatctgggcggcaaagtggcggatccgcagggcctgttttatagcagcccggaagaactgaaaagcctgggcgcgaacgtgcagatgaaccataacgtgctgaacattgatccggatcagaaaaccgtgaccgtggaaaacatgaacacccatgaacagaccaccgcggattatgataaactggtgatgaccagcggcagctggccgattgtgccgaaaattccgggcattgatggcgatcatgtgaaactgtgcaaaaactggaaccatgcgcagaccctgattgaagatgcgaaaagcgcgaaacatattaccgtgattggcgcgggctatattggcgcggaactggcggaagcgtatagcaccaccggccatgatgtgaccctgattgatgcgatggatcgcgtgatgccgaaatattttgatagcgaatttaccgatgtgattgaacaggattatcgcgataacaacgtgcagctggcgctgggcgaaaccgtgcagagctttaccgataccggcgatggcgtgaccattaaaaccgataaaggcagctatgataccaacctggcgattctgtgcattggctttcgcccgaacaccggcctgctgaaaggcaaagtggatatggcgaaaaacggcgcgattattaccgatgattatatgcgcagcagcaacccggatatttttgcggcgggcgatagcgcggcggtgcattataacccgacccatcagaacgcgtatattccgctggcgaccaacgcggtgcgccagggcattctggtgggcaaaaacctggtgaaaccgaccgtgaaatatatgggcacccagagcagcagcggcctggcgctgtatgatcgcaccattgtgagcaccggcctgaccctggcggcggcgaaacagcagggcattaacgcggaacaggtgattgtgaaagataactatcgcccggaatttatgccgaccaccgaaccggtgctgatgagcctggtgtttgatccggatagccgccgcattctgggcggcgcgctgatgagccgctatgatgtgagccagagcgcgaacaccctgagcgtgtgcattcagaacgaaaacaccattgatgatctggcgatggtggatatgctgtttcagccgaactttgatcgcccgtttaactatctgaacattctggcgcaggcggcgcaggaaaaagtggcgaaatttcagccggcggaataa

SEQ ID NO: 9 - protein, 510 aa, Vibrio harveyi
MNPQTDNVFYATNAFTGEALPLAFPVHTEVEVNQAATAAAKVARDFRRLNNSKRASLLRTIASELEARSDDIIARAHLETALPEVRLTGEIARTANQLRLFADVVNSGSYHQAILDTPNPTRAPLPKPDIRRQQIALGPVAVFGASNFPLAFSAAGGDTASALAAGCPVIVKGHTAHPGTSQIVAECIEQALKQEQLPQAIFTLLQGNQRALGQALVSHPEIKAVGFTGSVGGGRALFNLAHERPEPIPFYGELGAINPTFIFPSAMRAKADLADQFVASMTMGCGQFCTKPGVVFALNTPETQAFIETAQSLIRQQSPSTLLTPGIRDSYQSQVVSRGSDDGIDVTFSQAESPCVASALFVTSSENWRKHPAWEEEIFGPQSLIVVCENVADMLSLSEMLAGSLTATIHATEEDYPQVSQLIPRLEEIAGRLVFNGWPTGVEVGYAMVHGGPYPASTHSASTSVGAEAIHRWLRPVAYQALPESLLPDSLKAENPLEIARAVDGKAAHS

SEQ ID NO: 10 - protein, 510 aa, Vibrio harveyi
MNPQTDNVFYATNAFTGEALPLAFPVHTEVEVNQAATAAAKVARDFRRLNNSKRASLLRTIASELEARSDDIIARAHLETALPEVRLTGEIARTANQLRLFADVVNSGSYHQAILDTPNPTRAPLPKPDIRRQQIALGPVAVFGASNFPLAFSAAGGDTASALAAGCPVIVKGHQAHPGTSQIVAECIEQALKQEQLPQAIFTLLQGNQRALGQALVSHPEIKAVGFTGSVGGGRALFNLAHERPEPIPFYGELGAINPTFIFPSAMRAKADLADQFVASMTMGCGQFCTKPGVVFALNTPETQAFIETAQSLIRQQSPSTLLTPGIRDSYQSQVVSRGSDDGIDVTFSQAESPCVASALFVTSSENWRKHPAWEEEIFGPQSLIVVCENVADMLSLSEMLAGSLTATIHATEEDYPQVSQLIPRLEEIAGRLVFNGWPTGVEVGYAMVHGGPYPASTHSASTSVGAEAIHRWLRPVAYQALPESLLPDSLKAENPLEIARAVDGKAAHS

SEQ ID NO: 11 - protein, 507 aa, Rhodococcus erythropolis
MTVYARPGTADAIMSFQSRYDNWIGNEWVAPVKGQYFENPTPVTGQNFCDVARSTAEDIELALDAAHAAAPAWGKTSVAERAIILNKIADRMEENLESIALAESWDNGKPIRETLNADIPLAIDHFRYFAGAIRAQEGSLSEINSDTVAYHFHEPLGVVGQIIPWNFPILMAVWKLAPALAAGNAIVLKPAEQTPVSILHLIGIIGDLLPAGVLNIVNGFGVEAGKPLASSPRIKKIAFTGETTTGRLIMQYASQNLIPVTLELGGKSPNIFFSDVLASNDDYQDKALEGFTMFALNQGEVCTCPSRSLIQEDIFDEFLAMAAIRTKAVRQGDPLDTDTMIGAQASNDQLEKILSYIEIGKAEGAKVITGGERAELGGDLSGGYYVQPTVFTGNNKMRIFQEEIFGPVVSVTSFKDYDEAIEIANDTLYGLGAGVWSRDGGVAYRAGRDIQAGRVWTNTYHQYPAHAAFGGYKQSGIGRENHLMMLSHYQQTKNLLVSYAQKAQGFF

SEQ ID NO: 12 - protein, 506 aa, Geobacillus thermodenitrificans
MIYAQPGQPGALVTFKKRYENFIGGKWVPPVDGEYFENITPITGKPYCEVPRSKAADIELALDAAHAAKDEWGRTSPAKRARLLNKIADRMEENLELLAVAETWENGKPIRETLAADIPLAIDHFRYFASCIRAQEGTISEIDHDTVAYHFKEPLGVVGQIIPWNFPILMAAWKLAPALAAGNCVVLKPAEQTPTSILVLIELIEDLLPPGVVNIVNGFGLEAGKPLASNPRVAKVAFTGETTTGRLIMQYASQNIVPVTLELGGKSPNIFFADVMDKDDEFFDKALEGFTMFALNQGEVCTCPSRALIHESIYDAFMERALERVKQIKQGNPLDTETMIGAQASSEQLEKILSYIDIGKQEGAELLIGGERNMLEGELAGGYYVKPTIFKGHNKMRIFQEEIFGPVLAVTTFKDEDEALAIANETLYGLGAGVWTRNINTAYRFGRGIQAGRVWTNCYHVYPAHAAFGGYKMSGIGRETHKMMLDHYQQTKNMLVSYSPKKLGLF

SEQ ID NO: 13 - protein, 506 aa, Marinobacter aquaeolei
MIYAQPGQEGSVVSFKSRYENYIGGEWVAPVKGQYFDNITPVTGAVFCEVPRSTAEDIDLALDAAHKAAPAWGKTSPTERSNILLKIADRIEANLEKLAVAETWDNGKAVRETLNADVPLAADHLRYFAGCIRAQEGHMSEIDHNTVAYHFHEPLGVVGQIIPWNFPLLMAAWKLGPCLASGNCTVLKPAEQTPASILVLMDIIGDLLPPGVINIVNGYGIEAGQALATSKRIAKIAFTGSTPVGSHILKCAAENIIPSTVELGGKSPNIYFSDVMKAEPEFVDKCVEGLVLAFFNQGEICTCPSRALVQEDMFEEFMQKVVERTKSIKRGNPLDTDVQVGAQASKEQFDKIMSYMEIGRQEGAVVLTGGDREHLEGEFNNGFYIQPTLFKGDNKMRVFQEEIFGPVVGVTTFKTEEEALAIANDTEFGLGAGVWTRDTNLAYRMGRNIQAGRVWMNCYHAYPAHAAFGGYKKSGIGRENHKMALEHYQQTKCMLTSYDTNPLGFF

SEQ ID NO: 14 - protein, 503 aa, Acinebacter sp. Stamm M1
MHYVDPNQSGSKIHFKDQYENFIGGQWVAPVKGVYFDNISPVDGKSFTRIPRSSAEDIELALDAAHKAKKEWNKSSPTTRSNLLLKIADRMEANLEMLAVAETWDNGKPVRETLAADIPLAIDHFRYFAGCIRAQEGGISEIDEDTIAYHFHEPLGVVGQIIPWNFPILMAAWKLAPALAAGNCVVIKPAEQTPVGILLVAELIQDLLPAGVLNIVNGYGAEVGRPLATSPRIAKIAFTGSTQVGQLIMQYATENIIPVTLELGGKSPNVFFADVMDHDDDFLDKTLEGFAMFALNQGEVCTCPSRALIQESIADQFMEKAIERVKRIKLGHPLDTDTMVGAQASLEQQEKILRCIDTGRQEGAEVLLGGHGRQEVGNGYYIEPTIFKGHNNMQVFQEEIFGPVLSVTTFKDFDEAIQIANDTMYGLGAGVWSRSTHTAYRAGRAIEAGRVWTNCYHIYPAHAAFGGYKKSGVGRENHKMMLDHYQQTKNLLVSYSTKAMGFF

SEQ ID NO: 15 - protein, 529 aa, Yarrowia lipolytica
MTTTATETPTTNVTPTTSLPKETASPGGTASVNTSFDWESICGKTPLEEIESDISRLKKTFRSGKTLDLDYRLDQIRNLAYAIRDNENKIRDAIKADLKRPDFETMAAEFSVQMGEFNYVVKNLPKWVKDEKVKGTSMAYWNSSPKIRKRPLGSVLVITPWNYPLILAVSPVLGAIAAGNTVALKMSEMSPNASKVIGDIMTAALDPQLFQCFFGGVPETTEILKHRWDKIMYTGNGKVGRIICEAANKYLTPVELELGGKSPVFVTKHCSNLEMAARRIIWGKFVNGGQTCVAPDYVLVCPEVHDKFVAACQKVLDKFYPNNSAESEMAHIATPLHYERLTGLLNSTRGKVVAGGTFNSATRFIAPTIVDGVDANDSLMQGELFGPLLPIVKAMSTEAACNFVLEHHPTPLAEYIFSDNNSEIDYIRDRVSSGGLVINDTLIHVGCVQAPFGGVGDSGNGGYHGKHTFDLFSHSQTVLRQPGWVEMLQKKRYPPYNKSNEKFVRRMVVPSPGFPREGDVRGFWSRLFN